European Patent Specification EP 3 638 776 B1, published November 5, 2025. Title: Methods and means for genetic alteration of genomes utilizing designer DNA recombining enzymes. Applicant: Technische Universität Dresden. The sequence listing filed with the application follows.

SEQUENCE LISTING (49 sequences)

SEQ ID NO: 1 - protein, 343 aa, Artificial Sequence
  Recombinase F9-1
  MISC_FEATURE (17)..(17): Xaa can be any naturally occurring amino acid, preferably aspartic acid or glycine
  MISC_FEATURE (19)..(19): Xaa can be any naturally occurring amino acid, preferably threonine or alanine
  MISC_FEATURE (22)..(22): Xaa can be any naturally occurring amino acid, preferably glycine or glutamic acid
  MISC_FEATURE (30)..(30): Xaa is a small unpolar amino acid, preferably selected from valine, leucine, isoleucine, alanine and glycine
  MISC_FEATURE (43)..(43): Xaa is apositively charged amino acid, preferably lysine or arginine
  MISC_FEATURE (60)..(60): Xaa can be any naturally occurring amino acid, preferably aspartic acid or asparagine
  MISC_FEATURE (68)..(68): Xaa can be any naturally occurring amino acid, preferably proline or serine
  MISC_FEATURE (69)..(69): Xaa is a charged  amino acid, preferably selected form aspartic acid, glutamic acid, lysine or arginine
  MISC_FEATURE (81)..(81): Xaa is a polar amino acid, preferably selected from serine, threonine, cysteine, lysine or arginine
  MISC_FEATURE (84)..(84): Xaa can be any naturally occurring amino acid, preferably alanine or threonine
  MISC_FEATURE (89)..(89): Xaa can be any naturally occurring amino acid, preferably leucine or glutamine
  MISC_FEATURE (93)..(93): Xaa is a small amino acid, preferably selected from cysteine, serine and alanine
  MISC_FEATURE (140)..(140): Xaa can be any naturally occurring amino acid, preferably isoleucine or threonine
  MISC_FEATURE (166)..(166): Xaa is an unpolar amino acid, preferably selected from isoleucine, leucine and valine
  MISC_FEATURE (177)..(177): Xaa is an unpolar amino acid, preferably selected from isoleucine, leucine and valine
  MISC_FEATURE (182)..(182): Xaa is an unpolar amino acid, preferably selected from isoleucine, leucine and valine
  misc_feature (183)..(183): Xaa can be any naturally occurring amino acid
  MISC_FEATURE (184)..(184): Xaa is a postively cahrged amino acid, preferably selected from lysine and arginine
  MISC_FEATURE (186)..(186): Xaa is a polar amino acid, preferably selected from serine or threonine
  MISC_FEATURE (206)..(206): Xaa can be any naturally occurring amino acid, preferably alanine or threonine
  MISC_FEATURE (222)..(222): Xaa can be any naturally occurring amino acid, preferably valine or glutamic acid
  MISC_FEATURE (225)..(225): Xaa is an unpolar amino acid, preferably selected from isoleucine, leucine and valine
  MISC_FEATURE (237)..(237): Xaa is a polar amino acid, preferably selected from serine, threonine, cysteine or tyrosine
  MISC_FEATURE (239)..(239): Xaa is an unpolar amino acid, preferably selected from isoleucine, leucine, valine or phenylalanine
  MISC_FEATURE (249)..(249): Xaa is a small unpolar amino acid, preferably selected from alanine, glycine, isoleucine, leucine and valine
  MISC_FEATURE (259)..(259): Xaa can be any naturally occurring amino acid, preferably phenylalanine or proline
  MISC_FEATURE (260)..(260): Xaa can be any naturally occurring amino acid, preferably threonine or alanine
  MISC_FEATURE (264)..(264): Xaa can be any naturally occurring amino acid, preferably alanine or aspartic acid
  MISC_FEATURE (278)..(278): Xaa can be any naturally occurring amino acid, preferably leucine or glutamine
  MISC_FEATURE (284)..(284): Xaa is an unpolar amino acid, preferably selected from isoleucine, leucine or valine
  MISC_FEATURE (318)..(318): Xaa is an unpolar amino acid, preferably selected from isoleucine, leucine or valine
  MISC_FEATURE (342)..(342): Xaa can be any naturally occurring amino acid, preferably glycine or aspartic acid
MSNLQTLHQNLSALLVXAXSDXARKNLMDXFRDRQAFSEHTWXVLLSVCRSWAAWCKLNXRKWFPAEXXDVRDYLLHLQAXGLXVNTIXQHLXQLNMLHRRSGLPRPGDSNAVSLVMRRIRKENVDAGERVKQALAFERXDFDQVRSLMENSDRCQDIRNLAFLGXAYNTLLRISEXARIRXXDIXRTDGGRMLIHIGRTKTLVSXAGVEKALSLRVTRLVXRWXSVSGVADDPNNXLXCRVRRNGVAXPSATSQLSTXXLQGXFAAAHRLIYGARDXSGQRYXTWSGHSARVGAARDMARAGVSIAEIMQAGGWTTXESVMNYIRNLDSETGAMVRLLEDXD

SEQ ID NO: 2 - protein, 343 aa, Artificial Sequence
  Recombinase F9-2
  misc_feature (3)..(3): Xaa can be any naturally occurring amino acid
  misc_feature (5)..(5): Xaa can be any naturally occurring amino acid
  misc_feature (8)..(8): Xaa can be any naturally occurring amino acid
  misc_feature (14)..(14): Xaa can be any naturally occurring amino acid
  misc_feature (16)..(16): Xaa can be any naturally occurring amino acid
  misc_feature (18)..(21): Xaa can be any naturally occurring amino acid
  misc_feature (31)..(31): Xaa can be any naturally occurring amino acid
  misc_feature (39)..(39): Xaa can be any naturally occurring amino acid
  misc_feature (80)..(80): Xaa can be any naturally occurring amino acid
  misc_feature (84)..(84): Xaa can be any naturally occurring amino acid
  misc_feature (93)..(93): Xaa can be any naturally occurring amino acid
  misc_feature (97)..(97): Xaa can be any naturally occurring amino acid
  misc_feature (125)..(125): Xaa can be any naturally occurring amino acid
  misc_feature (132)..(132): Xaa can be any naturally occurring amino acid
  misc_feature (182)..(183): Xaa can be any naturally occurring amino acid
  misc_feature (186)..(186): Xaa can be any naturally occurring amino acid
  misc_feature (195)..(195): Xaa can be any naturally occurring amino acid
  misc_feature (206)..(206): Xaa can be any naturally occurring amino acid
  misc_feature (216)..(216): Xaa can be any naturally occurring amino acid
  misc_feature (249)..(249): Xaa can be any naturally occurring amino acid
  misc_feature (253)..(253): Xaa can be any naturally occurring amino acid
  misc_feature (259)..(260): Xaa can be any naturally occurring amino acid
  misc_feature (264)..(264): Xaa can be any naturally occurring amino acid
  misc_feature (266)..(266): Xaa can be any naturally occurring amino acid
  misc_feature (273)..(273): Xaa can be any naturally occurring amino acid
  misc_feature (276)..(276): Xaa can be any naturally occurring amino acid
  misc_feature (278)..(278): Xaa can be any naturally occurring amino acid
  misc_feature (306)..(306): Xaa can be any naturally occurring amino acid
  misc_feature (325)..(325): Xaa can be any naturally occurring amino acid
MSXLXTLXQNLSAXLXDXXXXEARKNLMDVXRDRQAFSXHTWRVLLSVCRSWAAWCELNNRKWFPAEPEDVRDYLLHLQXRGLXVNTIQQHLXQLNXLHRRSGLPRPGDSNAVSLVMRRIRKENXDAGERVXQALAFERTDFDQVRSLMENSDRCQDIRNLAFLGVAYNTLLRISEIARIRXXDIXRTDGGRMLXHIGRTKTLVSXAGVEKALSLXVTKLVERWISVSGVADDPNNYLFCRVRRNGVAXPSAXSQLSTXXLQGXFXAAHRLIXGAXDXSGQRYLTWSGHSARVGAARDMARAGVSXAEIMQAGGWTTVESVMNYXRNLDSETGAMVRLLEDGD

SEQ ID NO: 3 - protein, 343 aa, Artificial Sequence
  Recombinase F9-1a
MSNLQTLHQNLSALLVDATSDGARKNLMDVFRDRQAFSEHTWKVLLSVCRSWAAWCKLNNRKWFPAEPEDVRDYLLHLQACGLAVNTILQHLAQLNMLHRRSGLPRPGDSNAVSLVMRRIRKENVDAGERVKQALAFERIDFDQVRSLMENSDRCQDIRNLAFLGIAYNTLLRISEVARIRIKDISRTDGGRMLIHIGRTKTLVSAAGVEKALSLRVTRLVVRWVSVSGVADDPNNYLFCRVRRNGVAVPSATSQLSTFTLQGVFAAAHRLIYGARDASGQRYLTWSGHSARVGAARDMARAGVSIAEIMQAGGWTTVESVMNYIRNLDSETGAMVRLLEDGD

SEQ ID NO: 4 - protein, 343 aa, Artificial Sequence
  Recombinase F9-2a
MSKLPTLHQNLSALLADATSDEARKNLMDVLRDRQAFSKHTWRVLLSVCRSWAAWCELNNRKWFPAEPEDVRDYLLHLQTRGLTVNTIQQHLCQLNLLHRRSGLPRPGDSNAVSLVMRRIRKENIDAGERVKQALAFERTDFDQVRSLMENSDRCQDIRNLAFLGVAYNTLLRISEIARIRVRDITRTDGGRMLIHIGRTKTLVSAAGVEKALSLGVTKLVERWISVSGVADDPNNYLFCRVRRNGVAAPSAISQLSTPALQGVFAAAHRLIHGAKDASGQRYLTWSGHSARVGAARDMARAGVSVAEIMQAGGWTTVESVMNYLRNLDSETGAMVRLLEDGD

SEQ ID NO: 5 - protein, 343 aa, Artificial Sequence
  Recombinase F9-1b
MSNLQTLHQNLSALLVGAASDEARKNLMDAFRDRQAFSEHTWRVLLSVCRSWAAWCKLNDRKWFPAESKDVRDYLLHLQARGLTVNTIQQHLCQLNMLHRRSGLPRPGDSNAVSLVMRRIRKENVDAGERVKQALAFERTDFDQVRSLMENSDRCQDIRNLAFLGVAYNTLLRISEIARIRVRDITRTDGGRMLIHIGRTKTLVSTAGVEKALSLRVTRLVERWISVSGVADDPNNCLICRVRRNGVAAPSATSQLSTPALQGIFAAAHRLIYGARDDSGQRYQTWSGHSARVGAARDMARAGVSIAEIMQAGGWTTIESVMNYLRNLDSETGAMVRLLEDDD

SEQ ID NO: 6 - protein, 343 aa, Artificial Sequence
  F9-2b
MSNLQTLTQNLSAILVDGANGEARKNLMDVFRDRQAFSEHTWRVLLSVCRSWAAWCELNNRKWFPAEPEDVRDYLLHLQARGLAVNTIQQHLAQLNMLHRRSGLPRPGDSNAVSLVMRRIRKENVDAGERVRQALAFERTDFDQVRSLMENSDRCQDIRNLAFLGVAYNTLLRISEIARIRIKDISRTDGGRMLVHIGRTKTLVSTAGVEKALSLRVTKLVERWISVSGVADDPNNYLFCRVRRNGVAVPSATSQLSTSTLQGIFGAAHRLIYGAQDDSGQRYLTWSGHSARVGAARDMARAGVSIAEIMQAGGWTTVESVMNYIRNLDSETGAMVRLLEDGG

SEQ ID NO: 7 - DNA, 34 bp, Homo sapiens
ctcattacatttaaccaaaattatcacaatataa

SEQ ID NO: 8 - DNA, 34 bp, Homo sapiens
ccatcttttgttagatttgaatatatacattcta

SEQ ID NO: 9 - DNA, 34 bp, Bacteriophage P1
ataacttcgtataatgtatgctatacgaagttat

SEQ ID NO: 10 - DNA, 34 bp, Homo sapiens
atatatacgtatatagacatatatacgtatatat

SEQ ID NO: 11 - DNA, 34 bp, Artificial Sequence
  LoxM7 target site - artificial variant of LoxP
ataactctatataatgtatgctatatagagttat

SEQ ID NO: 12 - DNA, 34 bp, Artificial Sequence
  LoxM5 target site - artificial variant of LoxP
ataacttcgtgcaatgtatgctgcacgaagttat

SEQ ID NO: 13 - DNA, 34 bp, Human immunodeficiency virus
acaacatcctattacaccctatatgccaacatgg

SEQ ID NO: 14 - DNA, 34 bp, Human immunodeficiency virus
aacccactgcttaagcctcaataaagcttgcctt

SEQ ID NO: 15 - DNA, 34 bp, Artificial Sequence
  Intermediate target site loxF9-AL
ctcattacatttaaccaaaattaaatgtaatgag

SEQ ID NO: 16 - DNA, 34 bp, Artificial Sequence
  Intermediate target site loxF9-AR
ttatattgtgataaccaaaattatcacaatataa

SEQ ID NO: 17 - DNA, 34 bp, Artificial Sequence
  Intermediate target site loxF9-BLS
ccaacttttgatagatttgaatatcaaaagttgg

SEQ ID NO: 18 - DNA, 34 bp, Artificial Sequence
  Intermediate target site loxF9-BRS
tagactttatatagatttgaatatataaagtcta

SEQ ID NO: 19 - DNA, 34 bp, Artificial Sequence
  Intermediate target site loxF9-BL
ccatcttttgttagatttgaataacaaaagatgg

SEQ ID NO: 20 - DNA, 34 bp, Artificial Sequence; identical to SEQ ID NO: 19
  Intermediate target site loxF9-BR

SEQ ID NO: 21 - DNA, 7184 bp, Artificial Sequence
  vector pDuoF9 (source)
  P1 binding site (1412)..(1430)
  Rec. F9-1 (placeholder) (1519)..(2550)
  Ribosome binding site (2551)..(2633)
  Rec. F9-2 (placeholder) (2634)..(3665)
  LoxF9a (4220)..(4253)
  LoxF9b (4961)..(4994)
  P2 binding site (5012)..(5028)
  CmR (5315)..(5974)
  Ori (6336)..(7184)
gctcatgagcccgaagtggcgagcccgatcttccccatcggtgatgtcggcgatataggcgccagcaaccgcacctgtggcgccggtgatgccggccacgatgcgtccggcgtagaggatctgctcatgtttgacagcttatcatcgatgcataatgtgcctgtcaaatggacgaagcagggattctgcaaaccctatgctactccgtcaagccgtcaattgtctgattcgttaccaattatgacaacttgacggctacatcattcactttttcttcacaaccggcacggaactcgctcgggctggccccggtgcattttttaaatacccgcgagaaatagagttgatcgtcaaaaccaacattgcgaccgacggtggcgataggcatccgggtggtgctcaaaagcagcttcgcctggctgatacgttggtcctcgcgccagcttaagacgctaatccctaactgctggcggaaaagatgtgacagacgcgacggcgacaagcaaacatgctgtgcgacgctggcgatatcaaaattgctgtctgccaggtgatcgctgatgtactgacaagcctcgcgtacccgattatccatcggtggatggagcgactcgttaatcgcttccatgcgccgcagtaacaattgctcaagcagatttatcgccagcagctccgaatagcgcccttccccttgcccggcgttaatgatttgcccaaacaggtcgctgaaatgcggctggtgcgcttcatccgggcgaaagaaccccgtattggcaaatattgacggccagttaagccattcatgccagtaggcgcgcggacgaaagtaaacccactggtgataccattcgcgagcctccggatgacgaccgtagtgatgaatctctcctggcgggaacagcaaaatatcacccggtcggcaaacaaattctcgtccctgatttttcaccaccccctgaccgcgaatggtgagattgagaatataacctttcattcccagcggtcggtcgataaaaaaatcgagataaccgttggcctcaatcggcgttaaacccgccaccagatgggcattaaacgagtatcccggcagcaggggatcattttgcgcttcagccatacttttcatactcccgccattcagagaagaaaccaattgtccatattgcatcagacattgccgtcactgcgtcttttactggctcttctcgctaaccaaaccggtaaccccgcttattaaaagcattctgtaacaaagcgggaccaaagccatgacaaaaacgcgtaacaaaagtgtctataatcacggcagaaaagtccacattgattatttgcacggcgtcacactttgctatgccatagcatttttatccataagattagcggatcctacctgacgctttttatcgcaactctctactgtttctccatacccgtttttttgggctagcgaattcgagctctaaggaggtgccacaattctcgagccatacccattctaatgatcataaggaggtgtacatgtcaatactactgaccttgcaccaaagtttgtccgcattactggtcgatgcaacgagtgatgaggctcgcaagaacctgatggatgtgctcagggatcgccaggcgttctccgagcgtacctggaaagtgctcctgtccgtttgccggacgtgggcggcatggtgcaagttgaacaaccggaaatggtttcccgcggaacctgaagatgttcgcgattaccttctacatcttcaggctcgcggtctggcagtaaacactatcctgcaacatttggcccagctaaacatgctccaccgtcggttcgggctgccacgaccgggcgacagcgacgctgtttcactggttatgcggcgaatccgaagggagaacgtcgatgctggtgagcgtacgaagcaggccctagcgttcgagcgcactgacttcgaccaggttcgtgcactcatggaaaatagcgaacggggccaggatatacgtactctggcacttctgggggttgcttataacaccctgttacgcgtatccgaaattgccaggattcggattaaagacatctcacgtactgacggtgggaggatgctaatccacattagcagaacgaaaacgctggtcagcaccgcaggcgtagagaaggcgcttagcctgggggtaactaaactggtcgagcgatggatttccgtctctggtgtggctagtgacccaaacaattacctgttttgccaggttagaataaatggtgtggccgtgccgtctgccaccagccggctatcaaccgacgtcctgcgaaagatttttgaggctgcccaccgcctgatctacggtgccaaggatggctctggtcagagatacctggcctggtctgggcacagtgcccgtgtcggagccgcgcgggatatggcccgcgctggggtttcaatagcggagattatgcaggctggtggctggaccaccgtagagagtgtcatgaactatatccgtaacctggacagtgagacaggggcaatggtgcgtctgctggaagatggcgactagtctagaggtaccattccgatcgcggatcggccggaatgggatagacgtcctatcatccacacctactagttaaggaggtgtacatgtcaatactactgaccttgcaccaaagtttgtccgcattactggtcgatgcaacgagtgatgaggctcgcaagaacctgatggatgtgctcagggatcgccaggcgttctccgagcgtacctggaaagtgctcctgtccgtttgccggacgtgggcggcatggtgcaagttgaacaaccggaaatggtttcccgcggaacctgaagatgttcgcgattaccttctacatcttcaggctcgcggtctggcagtaaacactatcctgcaacatttggcccagctaaacatgctccaccgtcggttcgggctgccacgaccgggcgacagcgacgctgtttcactggttatgcggcgaatccgaagggagaacgtcgatgctggtgagcgtacgaagcaggccctagcgttcgagcgcactgacttcgaccaggttcgtgcactcatggaaaatagcgaacggggccaggatatacgtactctggcacttctgggggttgcttataacaccctgttacgcgtatccgaaattgccaggattcggattaaagacatctcacgtactgacggtgggaggatgctaatccacattagcagaacgaaaacgctggtcagcaccgcaggcgtagagaaggcgcttagcctgggggtaactaaactggtcgagcgatggatttccgtctctggtgtggctagtgacccaaacaattacctgttttgccaggttagaataaatggtgtggccgtgccgtctgccaccagccggctatcaaccgacgtcctgcgaaagatttttgaggctgcccaccgcctgatctacggtgccaaggatggctctggtcagagatacctggcctggtctgggcacagtgcccgtgtcggagccgcgcgggatatggcccgcgctggggtttcaatagcggagattatgcaggctggtggctggaccaccgtagagagtgtcatgaactatatccgtaacctggacagtgagacaggggcaatggtgcgtctgctggaagatggcgactagtctagacgtacgcctgcaggcaagcttggctgttttggcggatgagagaagattttcagcctgatacagattaaatcagaacgcagaagcggtctgataaaacagaatttgcctggcggcagtagcgcggtggtcccacctgaccccatgccgaactcagaagtgaaacgccgtagcgccgatggtagtgtggggtctccccatgcgagagtagggaactgccaggcatcaaataaaacgaaaggctcagtcgaaagactgggcctttcgttttatctgttgtttgtcggtgaacgctctcctgagtaggacaaatccgccgggagcggatttgaacgttgcgaagcaacggcccggagggtggcgggcaggacgcccgccataaactgccaggcatcaaattaagcagaaggccatcctgacggatggcctttttgcgtttctacaaactcttttgtttatttttctaaatacattcaaatatgtatccgctcatgagacaataaccctgataaatgcttcaataatattgaaaaaggaagagtatgagatctctcattacatttaaccaaaattatcacaatataaaagcttgcatgcctgcagatcgaggctggcctgtatcggacgggtcatctcgtttccttagctgtgtgcgccatgtaaatggcccggacgtgatggcgtaaatccacggctgtagcgcgctacgcttagatcctcatatggtgcactctcagtacaatctgctctgatgccgcatagttaagccagtatacactccgctatcgctacgtgactgggtcatggctgcgccccgacacccgccaacacccgctgacgcgccctgacgggcttgtctgctcccggcatccgcttacagacaagctgtgaccgtctccgggagctgcatgtgtcagaggttttcaccgtcatcaccgaaacgcgcgaggcagctgtggaatgtgtgtcagttagggtgtggaaagtccccaggctccccagcaggcagaagtatgcaaagcatgcatctcaattagtcagcaaccaggtgtggaaagtccccaggctccccagcaggcagaagtatgcaaagcatgcatctcaattagtcagcaaccatagtcccgcccctaactccgcccatcccgcccctaactccgcccagttccgcccattctccgccccatggctgactaattttttttatttatgcagaggccgaggccgcctcggcctaggaacagtcgacgacactgcagagacctacttcactaacaaccggtacagttcgaccatcttttgttagatttgaatatatacattctaagatctcaacatttccgtgtcgcccttattcccttttttgcggcattttgccttcctgtttttgctcacccagaaacgctggtgaaagtaaaagatgctgaagatcagttgggtgcagcaaactattaactggcgaactacttactctagcttcccggcaacaattaatagactggatggaggcggataaagttgcaggaccacttctgcgctcggcccggtcgaatttgctttcgaatttctgccattcatccgcttattatcacttattcaggcgtagcaccaggcgtttaagggcaccaataactgccttaaaaaaattacgccccgccctgccactcatcgcagtactgttgtaattcattaagcattctgccgacatggaagccatcacagacggcatgatgaacctgaatcgccagcggcatcagcaccttgtcgccttgcgtataatatttgcccatggtgaaaacgggggcgaagaagttgtccatattggccacgtttaaatcaaaactggtgaaactcacccagggattggctgagacgaaaaacatattctcaataaaccctttagggaaataggccaggttttcaccgtaacacgccacatcttgcgaatatatgtgtagaaactgccggaaatcgtcgtggtattcactccagagcgatgaaaacgtttcagtttgctcatggaaaacggtgtaacaagggtgaacactatcccatatcaccagctcaccgtctttcattgccatacggaattccggatgagcattcatcaggcgggcaagaatgtgaataaaggccggataaaacttgtgcttatttttctttacggtctttaaaaaggccgtaatatccagctgaacggtctggttataggtacattgagcaactgactgaaatgcctcaaaatgttctttacgatgccattgggatatatcaacggtggtatatccagtgatttttttctccattttagcttccttagctcctgaaaatctcgataactcaaaaaatacgcccggtagtgatcttatttcattatggtgaaagttggaacctcttacgtgccgatcaacgtctcattttcgccaaaagttggcccagggcttcccggtatcaacagggacaccaggatttatttattctgcgaagtgatcttccgtcacaggtatttattcggcgcaaagtgcgtcgggtgatgctgccaacttactgatttagtgtatgatggtgtttttgaggtgctccagtggcttctgtttctatcagctgtccctcctgttcagctactgacggggtggtgcgtaacggcaaaagcaccgccggacatcagcgctagcggagtgtatactggcttactatgttggcactgatgagggtgtcagtgaagtgcttcatgtggcaggagaaaaaaggctgcaccggtgcgtcagcagaatatgtgatacaggatatattccgcttcctcgctcactgactcgctacgctcggtcgttcgactgcggcgagcggaaatggcttacgaacggggcggagatttcctggaagatgccaggaagatacttaacagggaagtgagagggccgcggcaaagccgtttttccataggctccgcccccctgacaagcatcacgaaatctgacgctcaaatcagtggtggcgaaacccgacaggactataaagataccaggcgtttccccctggcggctccctcgtgcgctctcctgttcctgcctttcggtttaccggtgtcattccgctgttatggccgcgtttgtctcattccacgcctgacactcagttccgggtaggcagttcgctccaagctggactgtatgcacgaaccccccgttcagtccgaccgctgcgccttatccggtaactatcgtcttgagtccaacccggaaagacatgcaaaagcaccactggcagcagccactggtaattgatttagaggagttagtcttgaagtcatgcgccggttaaggctaaactgaaaggacaagttttggtgactgcgctcctccaagccagttacctcggttcaaagagttggtagctcagagaaccttcgaaaaaccgccctgcaaggcggttttttcgttttcagagcaagagattacgcgcagaccaaaacgatctcaagaagatcatcttattaatcagataaaatatttctag

SEQ ID NO: 22 - DNA, 2795 bp, Artificial Sequence
  pDonor vector
  AmpR (121)..(981)
  LoxF9a (1042)..(1075)
  KanR (1172)..(1987)
  LoxF9b (2062)..(2095)
  R6K-ori (2328)..(2719)
tttcggggaaatgtgcgcggaacccctatttgtttatttttctaaatacattcaaatatgtatccgctcatgagacaataaccctgataaatgcttcaataatattgaaaaaggaagagtatgagtattcaacatttccgtgtcgcccttattcccttttttgcggcattttgccttcctgtttttgctcacccagaaacgctggtgaaagtaaaagatgctgaagatcagttgggtgcacgagtgggttacatcgaactggatctcaacagcggtaagatccttgagagttttcgccccgaagaacgttttccaatgatgagcacttttaaagttctgctatgtggcgcggtattatcccgtgttgacgccgggcaagagcaactcggtcgccgcatacactattctcagaatgacttggttgagtactcaccagtcacagaaaagcatcttacggatggcatgacagtaagagaattatgcagtgctgccataaccatgagtgataacactgcggccaacttacttctgacaacgatcggaggaccgaaggagctaaccgcttttttgcacaacatgggggatcatgtaactcgccttgatcgttgggaaccggagctgaatgaagccataccaaacgacgagcgtgacaccacgatgcctgcagcaatggcaacaacgttgcgcaaactattaactggcgaactacttactctagcttcccggcaacaattaatagactggatggaggcggataaagttgcaggaccacttctgcgctcggcccttccggctggctggtttattgctgataaatctggagccggtgagcgtgggtctcgcggtatcattgcagcactggggccagatggtaagccctcccgtatcgtagttatctacacgacggggagtcaggcaactatggatgaacgaaatagacagatcgctgagataggtgcctcactgattaagcattggtaacccagcccgcctaatgagcgggcttttttttgaacaaaaggctgcagctggacttctagactcattacatttaaccaaaattatcacaatataaggtctgacgctcagtggaacgaaaactcacgttaagggattttggtcatgaacaataaaactgtctgcttacataaacagtaatacaaggggtgttatgagccatattcaacgggaaacgtcttgctctaggccgcgattaaattccaacatggatgctgatttatatgggtataaatgggctcgcgataatgtcgggcaatcaggtgcgacaatctatcgattgtatgggaagcccgatgcgccagagttgtttctgaaacatggcaaaggtagcgttgccaatgatgttacagatgagatggtcagactaaactggctgacggaatttatgcctcttccgaccatcaagcattttatccgtactcctgatgatgcatggttactcaccactgcgatccccgggaaaacagcattccaggtattagaagaatatcctgattcaggtgaaaatattgttgatgcgctggcagtgttcctgcgccggttgcattcgattcctgtttgtaattgtccttttaacagcgatcgcgtatttcgtctcgctcaggcgcaatcacgaatgaataacggtttggttgatgcgagtgattttgatgacgagcgtaatggctggcctgttgaacaagtctggaaagaaatgcataaacttttgccattctcaccggattcagtcgtcactcatggtgatttctcacttgataaccttatttttgacgaggggaaattaataggttgtattgatgttggacgagtcggaatcgcagaccgataccaggatcttgccatcctatggaactgcctcggtgagttttctccttcattacagaaacggctttttcaaaaatatggtgttgataatcctgatatgaataaattgcagtttcatttgatgctcgatgagtttttctaagaattaattcatgagcggatacatatttgaatgtatttagaaaaataaacaaataggggttccgcgcacatttcccatcttttgttagatttgaatatatacattctactcgagggtgcgaataagggacatgaagaaggaacacccgctcgcgggtgggcctacttcacctatcctgcccggctgacgccgttggatacaccaaggaaagtctacacgaaccctttggcaaaatcctgtatatcgtgcgaaaaaggatggatataccgaaaaaatcgctataatgaccccgaagcagggttatgcagcggaaaacggccacgatgcgtccggcgtagaggatctgaagatcagcagttcaacctgttgatagtacgtactaagctctcatgtttcacgtactaagctctcatgtttaacgtactaagctctcatgtttaacgaactaaaccctcatggctaacgtactaagctctcatggctaacgtactaagctctcatgtttcacgtactaagctctcatgtttgaacaataaaattaatataaatcagcaacttaaatagcctctaaggttttaagttttataagaaaaaaaagaatatataaggcttttaaagcttttaaggtttaacggttgtggacaacaagccagggatgtaacgcactgagaagcccttagagcctctcaaagcaattttgagtgacacaggaacacttaacggctgacatgggaattagcttcacgctgccgcaagcactcagggcgcaagggctgctaaaggaagcggatagacgtcaggtggcact

SEQ ID NO: 23 - DNA, 19 bp, Artificial Sequence
  Primer P1 for amplifying the plasmid pDuoF9
ctctactgtttctccatac

SEQ ID NO: 24 - DNA, 17 bp, Artificial Sequence
  Primer P2 for amplifying the plasmid pDuoF9
agggaataagggcgaca

SEQ ID NO: 25 - DNA, 7463 bp, Artificial Sequence
  vector pDuoF9 product
  P1 binding site (1412)..(1430)
  Rec. F9-1 (placeholder) (1519)..(2550)
  Ribosome binding site (2551)..(2633)
  Rec. F9-2 (placeholder) (2634)..(3665)
  LoxF9a (4220)..(4253)
  KanR (4350)..(5165)
  LoxF9b (5240)..(5273)
  P2 binding site (5291)..(5307)
  CmR (5594)..(6253)
  Ori (6615)..(7463)
gctcatgagcccgaagtggcgagcccgatcttccccatcggtgatgtcggcgatataggcgccagcaaccgcacctgtggcgccggtgatgccggccacgatgcgtccggcgtagaggatctgctcatgtttgacagcttatcatcgatgcataatgtgcctgtcaaatggacgaagcagggattctgcaaaccctatgctactccgtcaagccgtcaattgtctgattcgttaccaattatgacaacttgacggctacatcattcactttttcttcacaaccggcacggaactcgctcgggctggccccggtgcattttttaaatacccgcgagaaatagagttgatcgtcaaaaccaacattgcgaccgacggtggcgataggcatccgggtggtgctcaaaagcagcttcgcctggctgatacgttggtcctcgcgccagcttaagacgctaatccctaactgctggcggaaaagatgtgacagacgcgacggcgacaagcaaacatgctgtgcgacgctggcgatatcaaaattgctgtctgccaggtgatcgctgatgtactgacaagcctcgcgtacccgattatccatcggtggatggagcgactcgttaatcgcttccatgcgccgcagtaacaattgctcaagcagatttatcgccagcagctccgaatagcgcccttccccttgcccggcgttaatgatttgcccaaacaggtcgctgaaatgcggctggtgcgcttcatccgggcgaaagaaccccgtattggcaaatattgacggccagttaagccattcatgccagtaggcgcgcggacgaaagtaaacccactggtgataccattcgcgagcctccggatgacgaccgtagtgatgaatctctcctggcgggaacagcaaaatatcacccggtcggcaaacaaattctcgtccctgatttttcaccaccccctgaccgcgaatggtgagattgagaatataacctttcattcccagcggtcggtcgataaaaaaatcgagataaccgttggcctcaatcggcgttaaacccgccaccagatgggcattaaacgagtatcccggcagcaggggatcattttgcgcttcagccatacttttcatactcccgccattcagagaagaaaccaattgtccatattgcatcagacattgccgtcactgcgtcttttactggctcttctcgctaaccaaaccggtaaccccgcttattaaaagcattctgtaacaaagcgggaccaaagccatgacaaaaacgcgtaacaaaagtgtctataatcacggcagaaaagtccacattgattatttgcacggcgtcacactttgctatgccatagcatttttatccataagattagcggatcctacctgacgctttttatcgcaactctctactgtttctccatacccgtttttttgggctagcgaattcgagctctaaggaggtgccacaattctcgagccatacccattctaatgatcataaggaggtgtacatgtcaatactactgaccttgcaccaaagtttgtccgcattactggtcgatgcaacgagtgatgaggctcgcaagaacctgatggatgtgctcagggatcgccaggcgttctccgagcgtacctggaaagtgctcctgtccgtttgccggacgtgggcggcatggtgcaagttgaacaaccggaaatggtttcccgcggaacctgaagatgttcgcgattaccttctacatcttcaggctcgcggtctggcagtaaacactatcctgcaacatttggcccagctaaacatgctccaccgtcggttcgggctgccacgaccgggcgacagcgacgctgtttcactggttatgcggcgaatccgaagggagaacgtcgatgctggtgagcgtaccaagcaggccctagcgttcgagcgcactgacttcgaccaggttcgtgcactcatggaaaatagcgaacggggccaggatatacgtactctggcacttctgggggttgcttataacaccctgttacgcgtatccgaaattgccaggattcggattaaagacatctcacgtactgacggtgggaggatgctaatccacattagcagaacgaaaacgctggtcagcaccgcaggcgtagagaaggcgcttagcctgggggtaactaaactggtcgagcgatggatttccgtctctggtgtggctagtgacccaaacaattacctgttttgccaggttagaataaatggtgtggccgtgccgtctgccaccagccggctatcaaccgacgtcctgcgaaagatttttgaggctgcccaccgcctgatctacggtgccaaggatggctctggtcagagatacctggcctggtctgggcacagtgcccgtgtcggagccgcgcgggatatggcccgcgctggggtttcaatagcggagattatgcaggctggtggctggaccaccgtagagagtgtcatgaactatatccgtaacctggacagtgagacaggggcaatggtgcgtctgctggaagatggcgactagtctagaggtaccattccgatcgcggatcggccggaatgggatagacgtcctatcatccacacctactagttaaggaggtgtacatgtcaatactactgaccttgcaccaaagtttgtccgcattactggtcgatgcaacgagtgatgaggctcgcaagaacctgatggatgtgctcagggatcgccaggcgttctccgagcgtacctggaaagtgctcctgtccgtttgccggacgtgggcggcatggtgcaagttgaacaaccggaaatggtttcccgcggaacctgaagatgttcgcgattaccttctacatcttcaggctcgcggtctggcagtaaacactatcctgcaacatttggcccagctaaacatgctccaccgtcggttcgggctgccacgaccgggcgacagcgacgctgtttcactggttatgcggcgaatccgaagggagaacgtcgatgctggtgagcgtaccaagcaggccctagcgttcgagcgcactgacttcgaccaggttcgtgcactcatggaaaatagcgaacggggccaggatatacgtactctggcacttctgggggttgcttataacaccctgttacgcgtatccgaaattgccaggattcggattaaagacatctcacgtactgacggtgggaggatgctaatccacattagcagaacgaaaacgctggtcagcaccgcaggcgtagagaaggcgcttagcctgggggtaactaaactggtcgagcgatggatttccgtctctggtgtggctagtgacccaaacaattacctgttttgccaggttagaataaatggtgtggccgtgccgtctgccaccagccggctatcaaccgacgtcctgcgaaagatttttgaggctgcccaccgcctgatctacggtgccaaggatggctctggtcagagatacctggcctggtctgggcacagtgcccgtgtcggagccgcgcgggatatggcccgcgctggggtttcaatagcggagattatgcaggctggtggctggaccaccgtagagagtgtcatgaactatatccgtaacctggacagtgagacaggggcaatggtgcgtctgctggaagatggcgactagtctagacgtacgcctgcaggcaagcttggctgttttggcggatgagagaagattttcagcctgatacagattaaatcagaacgcagaagcggtctgataaaacagaatttgcctggcggcagtagcgcggtggtcccacctgaccccatgccgaactcagaagtgaaacgccgtagcgccgatggtagtgtggggtctccccatgcgagagtagggaactgccaggcatcaaataaaacgaaaggctcagtcgaaagactgggcctttcgttttatctgttgtttgtcggtgaacgctctcctgagtaggacaaatccgccgggagcggatttgaacgttgcgaagcaacggcccggagggtggcgggcaggacgcccgccataaactgccaggcatcaaattaagcagaaggccatcctgacggatggcctttttgcgtttctacaaactcttttgtttatttttctaaatacattcaaatatgtatccgctcatgagacaataaccctgataaatgcttcaataatattgaaaaaggaagagtatgagatctctcattacatttaaccaaaattatcacaatataaggtctgacgctcagtggaacgaaaactcacgttaagggattttggtcatgaacaataaaactgtctgcttacataaacagtaatacaaggggtgttatgagccatattcaacgggaaacgtcttgctctaggccgcgattaaattccaacatggatgctgatttatatgggtataaatgggctcgcgataatgtcgggcaatcaggtgcgacaatctatcgattgtatgggaagcccgatgcgccagagttgtttctgaaacatggcaaaggtagcgttgccaatgatgttacagatgagatggtcagactaaactggctgacggaatttatgcctcttccgaccatcaagcattttatccgtactcctgatgatgcatggttactcaccactgcgatccccgggaaaacagcattccaggtattagaagaatatcctgattcaggtgaaaatattgttgatgcgctggcagtgttcctgcgccggttgcattcgattcctgtttgtaattgtccttttaacagcgatcgcgtatttcgtctcgctcaggcgcaatcacgaatgaataacggtttggttgatgcgagtgattttgatgacgagcgtaatggctggcctgttgaacaagtctggaaagaaatgcataaacttttgccattctcaccggattcagtcgtcactcatggtgatttctcacttgataaccttatttttgacgaggggaaattaataggttgtattgatgttggacgagtcggaatcgcagaccgataccaggatcttgccatcctatggaactgcctcggtgagttttctccttcattacagaaacggctttttcaaaaatatggtgttgataatcctgatatgaataaattgcagtttcatttgatgctcgatgagtttttctaagaattaattcatgagcggatacatatttgaatgtatttagaaaaataaacaaataggggttccgcgcacatttcccatcttttgttagatttgaatatatacattctaagatctcaacatttccgtgtcgcccttattcccttttttgcggcattttgccttcctgtttttgctcacccagaaacgctggtgaaagtaaaagatgctgaagatcagttgggtgcagcaaactattaactggcgaactacttactctagcttcccggcaacaattaatagactggatggaggcggataaagttgcaggaccacttctgcgctcggcccggtcgaatttgctttcgaatttctgccattcatccgcttattatcacttattcaggcgtagcaccaggcgtttaagggcaccaataactgccttaaaaaaattacgccccgccctgccactcatcgcagtactgttgtaattcattaagcattctgccgacatggaagccatcacagacggcatgatgaacctgaatcgccagcggcatcagcaccttgtcgccttgcgtataatatttgcccatggtgaaaacgggggcgaagaagttgtccatattggccacgtttaaatcaaaactggtgaaactcacccagggattggctgagacgaaaaacatattctcaataaaccctttagggaaataggccaggttttcaccgtaacacgccacatcttgcgaatatatgtgtagaaactgccggaaatcgtcgtggtattcactccagagcgatgaaaacgtttcagtttgctcatggaaaacggtgtaacaagggtgaacactatcccatatcaccagctcaccgtctttcattgccatacggaattccggatgagcattcatcaggcgggcaagaatgtgaataaaggccggataaaacttgtgcttatttttctttacggtctttaaaaaggccgtaatatccagctgaacggtctggttataggtacattgagcaactgactgaaatgcctcaaaatgttctttacgatgccattgggatatatcaacggtggtatatccagtgatttttttctccattttagcttccttagctcctgaaaatctcgataactcaaaaaatacgcccggtagtgatcttatttcattatggtgaaagttggaacctcttacgtgccgatcaacgtctcattttcgccaaaagttggcccagggcttcccggtatcaacagggacaccaggatttatttattctgcgaagtgatcttccgtcacaggtatttattcggcgcaaagtgcgtcgggtgatgctgccaacttactgatttagtgtatgatggtgtttttgaggtgctccagtggcttctgtttctatcagctgtccctcctgttcagctactgacggggtggtgcgtaacggcaaaagcaccgccggacatcagcgctagcggagtgtatactggcttactatgttggcactgatgagggtgtcagtgaagtgcttcatgtggcaggagaaaaaaggctgcaccggtgcgtcagcagaatatgtgatacaggatatattccgcttcctcgctcactgactcgctacgctcggtcgttcgactgcggcgagcggaaatggcttacgaacggggcggagatttcctggaagatgccaggaagatacttaacagggaagtgagagggccgcggcaaagccgtttttccataggctccgcccccctgacaagcatcacgaaatctgacgctcaaatcagtggtggcgaaacccgacaggactataaagataccaggcgtttccccctggcggctccctcgtgcgctctcctgttcctgcctttcggtttaccggtgtcattccgctgttatggccgcgtttgtctcattccacgcctgacactcagttccgggtaggcagttcgctccaagctggactgtatgcacgaaccccccgttcagtccgaccgctgcgccttatccggtaactatcgtcttgagtccaacccggaaagacatgcaaaagcaccactggcagcagccactggtaattgatttagaggagttagtcttgaagtcatgcgccggttaaggctaaactgaaaggacaagttttggtgactgcgctcctccaagccagttacctcggttcaaagagttggtagctcagagaaccttcgaaaaaccgccctgcaaggcggttttttcgttttcagagcaagagattacgcgcagaccaaaacgatctcaagaagatcatcttattaatcagataaaatatttctag

SEQ ID NO: 26 - DNA, 800 bp, Homo sapiens
  loxF9a (1)..(34)
  loxF9b (766)..(800)
  Exon 8 of the F9 gene wildtype (766)..(800)
ctcattacatttaaccaaaattatcacaatataagaatgagatctttaacattgccaattaggtcagtggtcccaagtagtcacttagaaaatctgtgtatgtgaaatactgtttgtgacttaaaatgaaatttatttttaataggtgaacataatattgaggagacagaacatacagagcaaaagcgaaatgtgattcgaattattcctcaccacaactacaatgcagctattaataagtacaaccatgacattgcccttctggaactggacgaacccttagtgctaaacagctacgttacacctatttgcattgctgacaaggaatacacgaacatcttcctcaaatttggatctggctatgtaagtggctggggaagagtcttccacaaagggagatcagctttagttcttcagtaccttagagttccacttgttgaccgagccacatgtcttcgatctacaaagttcaccatctataacaacatgttctgtgctggcttccatgaaggaggtagagattcatgtcaaggagatagtgggggaccccatgttactgaagtggaagggaccagtttcttaactggaattattagctggggtgaagagtgtgcaatgaaaggcaaatatggaatatataccaaggtatcccggtatgtcaactggattaaggaaaaaacaaagctcacttaatgaaagatggatttccaaggttaattcattggaattgaaaattaacagggcctctcactaactaatcactttcccatcttttgttagatttgaatatatacattcta

SEQ ID NO: 27 - DNA, 800 bp, Homo sapiens
  loxF9a (1)..(34)
  Exon 8 of the F9 gene Arg338Leu (Padua mutation) (146)..(693)
  LoxF9b (766)..(800)
ctcattacatttaaccaaaattatcacaatataagaatgagatctttaacattgccaattaggtcagtggtcccaagtagtcacttagaaaatctgtgtatgtgaaatactgtttgtgacttaaaatgaaatttatttttaataggtgaacataatattgaggagacagaacatacagagcaaaagcgaaatgtgattcgaattattcctcaccacaactacaatgcagctattaataagtacaaccatgacattgcccttctggaactggacgaacccttagtgctaaacagctacgttacacctatttgcattgctgacaaggaatacacgaacatcttcctcaaatttggatctggctatgtaagtggctggggaagagtcttccacaaagggagatcagctttagttcttcagtaccttagagttccacttgttgaccgagccacatgtcttctgtctacaaagttcaccatctataacaacatgttctgtgctggcttccatgaaggaggtagagattcatgtcaaggagatagtgggggaccccatgttactgaagtggaagggaccagtttcttaactggaattattagctggggtgaagagtgtgcaatgaaaggcaaatatggaatatataccaaggtatcccggtatgtcaactggattaaggaaaaaacaaagctcacttaatgaaagatggatttccaaggttaattcattggaattgaaaattaacagggcctctcactaactaatcactttcccatcttttgttagatttgaatatatacattcta

SEQ ID NO: 28 - protein, 343 aa, Artificial Sequence; identical to SEQ ID NO: 1
  Recombinase F9-1
  misc_feature (17)..(17): Xaa can be any naturally occurring amino acid
  misc_feature (19)..(19): Xaa can be any naturally occurring amino acid
  misc_feature (22)..(22): Xaa can be any naturally occurring amino acid
  misc_feature (30)..(30): Xaa can be any naturally occurring amino acid
  misc_feature (43)..(43): Xaa can be any naturally occurring amino acid
  misc_feature (60)..(60): Xaa can be any naturally occurring amino acid
  misc_feature (68)..(69): Xaa can be any naturally occurring amino acid
  misc_feature (81)..(81): Xaa can be any naturally occurring amino acid
  misc_feature (84)..(84): Xaa can be any naturally occurring amino acid
  misc_feature (89)..(89): Xaa can be any naturally occurring amino acid
  misc_feature (93)..(93): Xaa can be any naturally occurring amino acid
  misc_feature (140)..(140): Xaa can be any naturally occurring amino acid
  misc_feature (166)..(166): Xaa can be any naturally occurring amino acid
  misc_feature (177)..(177): Xaa can be any naturally occurring amino acid
  misc_feature (182)..(183): Xaa can be any naturally occurring amino acid
  misc_feature (186)..(186): Xaa can be any naturally occurring amino acid
  misc_feature (206)..(206): Xaa can be any naturally occurring amino acid
  misc_feature (222)..(222): Xaa can be any naturally occurring amino acid
  misc_feature (225)..(225): Xaa can be any naturally occurring amino acid
  misc_feature (237)..(237): Xaa can be any naturally occurring amino acid
  misc_feature (239)..(239): Xaa can be any naturally occurring amino acid
  misc_feature (249)..(249): Xaa can be any naturally occurring amino acid
  misc_feature (259)..(260): Xaa can be any naturally occurring amino acid
  misc_feature (264)..(264): Xaa can be any naturally occurring amino acid
  misc_feature (278)..(278): Xaa can be any naturally occurring amino acid
  misc_feature (284)..(284): Xaa can be any naturally occurring amino acid
  misc_feature (318)..(318): Xaa can be any naturally occurring amino acid
  misc_feature (342)..(342): Xaa can be any naturally occurring amino acid

SEQ ID NO: 29 - protein, 343 aa, Artificial Sequence; identical to SEQ ID NO: 2
  Recombinase F9-1
  misc_feature (3)..(3): Xaa can be any naturally occurring amino acid
  misc_feature (5)..(5): Xaa can be any naturally occurring amino acid
  misc_feature (8)..(8): Xaa can be any naturally occurring amino acid
  misc_feature (14)..(14): Xaa can be any naturally occurring amino acid
  misc_feature (16)..(16): Xaa can be any naturally occurring amino acid
  misc_feature (18)..(21): Xaa can be any naturally occurring amino acid
  misc_feature (31)..(31): Xaa can be any naturally occurring amino acid
  misc_feature (39)..(39): Xaa can be any naturally occurring amino acid
  misc_feature (80)..(80): Xaa can be any naturally occurring amino acid
  misc_feature (84)..(84): Xaa can be any naturally occurring amino acid
  misc_feature (93)..(93): Xaa can be any naturally occurring amino acid
  misc_feature (97)..(97): Xaa can be any naturally occurring amino acid
  misc_feature (125)..(125): Xaa can be any naturally occurring amino acid
  misc_feature (132)..(132): Xaa can be any naturally occurring amino acid
  misc_feature (182)..(183): Xaa can be any naturally occurring amino acid
  misc_feature (186)..(186): Xaa can be any naturally occurring amino acid
  misc_feature (195)..(195): Xaa can be any naturally occurring amino acid
  misc_feature (206)..(206): Xaa can be any naturally occurring amino acid
  misc_feature (216)..(216): Xaa can be any naturally occurring amino acid
  misc_feature (249)..(249): Xaa can be any naturally occurring amino acid
  misc_feature (253)..(253): Xaa can be any naturally occurring amino acid
  misc_feature (259)..(260): Xaa can be any naturally occurring amino acid
  misc_feature (264)..(264): Xaa can be any naturally occurring amino acid
  misc_feature (266)..(266): Xaa can be any naturally occurring amino acid
  misc_feature (273)..(273): Xaa can be any naturally occurring amino acid
  misc_feature (276)..(276): Xaa can be any naturally occurring amino acid
  misc_feature (278)..(278): Xaa can be any naturally occurring amino acid
  misc_feature (306)..(306): Xaa can be any naturally occurring amino acid
  misc_feature (325)..(325): Xaa can be any naturally occurring amino acid

SEQ ID NO: 30 - DNA, 20 bp, Artificial Sequence
  Primer P1# for amplifying the plasmid pDuoF9
cggcgtcacactttgctatg

SEQ ID NO: 31 - DNA, 20 bp, Artificial Sequence
  Primer P2# for amplifying the plasmid pDuoF9
cccttaaacgcctggtgcta

SEQ ID NO: 32 - DNA, 20 bp, Artificial Sequence
  Primer P3 for amplifying the recombinase library
aagattagcggatcctacct

SEQ ID NO: 33 - DNA, 20 bp, Artificial Sequence
  Primer P4 for amplifying the recombinase library
gtgattagttagtgagaggc

SEQ ID NO: 34 - protein, 343 aa, Artificial Sequence
  Recombinase R#1
MSKLQTIHQNLSALLVDATSDEARKNLMDVLRDRQAFSKHTWRVLLSVCRSWAAWCELNNRKWFPAEPEDVRDYLLHLQTRGLTVNTIQQHLCQLNLLHRRSGLPRPGDSNAVSLVMRRIRKENIDAGERVKQALAFERTDFDQVRSLMENSDRCQDIRNLAFLGVAYNTLLRISEIARIRVRDITRTDGGRMLIHIGRTKTLVSAAGVEKALSLGVTKLVERWISVSGVADDPNNYLFCRVRRNGVAAPSAISQLSTPALQGVFAAAHRLIHGAKDASGQRYLTWSGHSARVGAARDMARAGVSVAEIMQAGGWTTVESVMNYLRNLDSETGAMVRLLEDGD

SEQ ID NO: 35 - protein, 343 aa, Artificial Sequence
  Recombinase R#7-B5
MSKLQTIHQDLSALLVDVTSDEARKNLMDVLRDRQAFSKHTWRVLLSVCRSWAAWCELNNRKWFPAEPEDVRDYLLHLQTRGLTVNTIQQHLCQLNLLHRRSGLPRPGDSNAVSLVMRRIRKENIDAGERVKQALAFERTDFDQVRSLMENSDRCQDIRNLAFLGVAYNTLLRISEIARIRVRDITRTDGGRMLIHIGRTKTLVSAAGVEKALSLGVTKLVERWISVSGVADDPNNHLFCRVRRNGVAAPSAISQLSTPALQGVFAAAHRLIHGAKDASGQRYLTWSGHSARVGAARDMARAGVSVAEIMQAGGWTTVESVMNYLRNLDSETGAMVRLLEDGD

SEQ ID NO: 36 - protein, 343 aa, Artificial Sequence
  Recombinase F9-3
MPKLQTIHQDLSALLVDVTSDEARKNLMDVLRDRQAFSRHTWRVLLSVCRSWAAWCELNNRKWFPAEPEDVRDYLLQLQTRGLTVNTIQQHLCQLNLLHRRSGLPRPGDSNAVSLVMRRIRKENIDAGERVKQALAFERTDFDQVRSLMENSDRCQDIRNLAFLGVAYNTLLRISEIARIRVRDITRTDGGRMLIHIGITKTLVSAAGVEKALSLGVTKLVERWISVSGVADDPNNHLFCRVRRNGVAAPSAISQLSTPALQGVFAAAHRLIHGAKDDSGQRYLTWSGHSARVGAARDMARAGVPVAEIMQAGGWTTVESVMSYLRNLDSETGAMVRLLEDGD

SEQ ID NO: 37 - DNA, 4930 bp, Artificial Sequence
  Plasmid pDonor-ex8
  Origin of replication (167)..(786)
  AmpR (941)..(1801)
  KanR (1822)..(2610)
  part of human F9 gene including exon 8 (3638)..(4636)
  LoxF9a (3713)..(3746)
  LoxF9b (4479)..(4512)
  P4 binding site (4479)..(4512)
cttccgcttcctcgctcactgactcgctgcgctcggtcgttcggctgcggcgagcggtatcagctcactcaaaggcggtaatacggttatccacagaatcaggggataacgcaggaaagaacatgtgagcaaaaggccagcaaaaggccaggaaccgtaaaaaggccgcgttgctggcgtttttccataggctccgcccccctgacgagcatcacaaaaatcgacgctcaagtcagaggtggcgaaacccgacaggactataaagataccaggcgtttccccctggaagctccctcgtgcgctctcctgttccgaccctgccgcttaccggatacctgtccgcctttctcccttcgggaagcgtggcgctttctcatagctcacgctgtaggtatctcagttcggtgtaggtcgttcgctccaagctgggctgtgtgcacgaaccccccgttcagcccgaccgctgcgccttatccggtaactatcgtcttgagtccaacccggtaagacacgacttatcgccactggcagcagccactggtaacaggattagcagagcgaggtatgtaggcggtgctacagagttcttgaagtggtggcctaactacggctacactagaagaacagtatttggtatctgcgctctgctgaagccagttaccttcggaaaaagagttggtagctcttgatccggcaaacaaaccaccgctggtagcggtggtttttttgtttgcaagcagcagattacgcgcagaaaaaaaggatctcaagaagatcctttgatcttttctacggggtctgacgctcagtggaacgaaaactcacgttaagggattttggtcatgagattatcaaaaaggatcttcacctagatccttttaaattaaaaatgaagttttaaatcaatctaaagtatatatgagtaaacttggtctgacagttaccaatgcttaatcagtgaggcacctatctcagcgatctgtctatttcgttcatccatagttgcctgactccccgtcgtgtagataactacgatacgggagggcttaccatctggccccagtgctgcaatgataccgcgagacccacgctcaccggctccagatttatcagcaataaaccagccagccggaagggccgagcgcagaagtggtcctgcaactttatccgcctccatccagtctattaattgttgccgggaagctagagtaagtagttcgccagttaatagtttgcgcaacgttgttgccattgctacaggcatcgtggtgtcacgctcgtcgtttggtatggcttcattcagctccggttcccaacgatcaaggcgagttacatgatcccccatgttgtgcaaaaaagcggttagctccttcggtcctccgatcgttgtcagaagtaagttggccgcagtgttatcactcatggttatggcagcactgcataattctcttactgtcatgccatccgtaagatgcttttctgtgactggtgagtactcaaccaagtcattctgagaatagtgtatgcggcgaccgagttgctcttgcccggcgtcaatacgggataataccgcgccacatagcagaactttaaaagtgctcatcattggaaaacgttcttcggggcgaaaactctcaaggatcttaccgctgttgagatccagttcgatgtaacccactcgtgcacccaactgatcttcagcatcttttactttcaccagcgtttctgggtgagcaaaaacaggaaggcaaaatgccgcaaaaaagggaataagggcgacacggaaatgttgaatactcatactcttcctttttcaattcagaagaactcgtcaagaaggcgatagaaggcgatgcgctgcgaatcgggagcggcgataccgtaaagcacgaggaagcggtcagcccattcgccgccaagctcttcagcaatatcacgggtagccaacgctatgtcctgatagcggtccgccacacccagccggccacagtcgatgaatccagaaaagcggccattttccaccatgatattcggcaagcaggcatcgccatgggtcacgacgagatcctcgccgtcgggcatgcgcgccttgagcctggcgaacagttcggctggcgcgagcccctgatgctcttcgtccagatcatcctgatcgacaagaccggcttccatccgagtacgtgctcgctcgatgcgatgtttcgcttggtggtcgaatgggcaggtagccggatcaagcgtatgcagccgccgcattgcatcagccatgatggatactttctcggcaggagcaaggtgggatgacaggagatcctgccccggcacttcgcccaatagcagccagtcccttcccgcttcagtgacaacgtcgagcacagctgcgcaaggaacgcccgtcgtggccagccacgatagccgcgctgcctcgtcctgcagttcattcagggcaccggacaggtcggtcttgacaaaaagaaccgggcgcccctgcgctgacagccggaacacggcggcatcagagcagccgattgtctgttgtgcccagtcatagccgaatagcctctccacccaagcggccggagaacctgcgtgcaatccatcttgttcaatcatgcgaaacgatcctcatcctgtctcttgatcagatcttgatcccctgcgccatcagatccttggcggcaagaaagccatccagtttactttgcagggcttcccaaccttaccagagggcgccccagctggcaattccggttcgcttgctgtccataaaaccgcccagtctagctatcgccatgtaagcccactgcaagctacctgctttctctttgcgcttgcgttttcccttgtccagatagcccagtagctgacattcatccggggtcagcaccgtttctgcggactggctttctacgtgttccgcttcctttagcagcccttgcgccctgaattttgttaaaattcgcgttaaatttttgttaaatcagctcattttttaaccaataggccgaaatcggcaaaatcccttataaatcaaaagaatagaccgagatagggttgagtgttgttccagtttggaacaagagtccactattaaagaacgtggactccaacgtcaaagggcgaaaaaccgtctatcagggcgatggcccactacgtgaaccatcaccctaatcaagttttttggggtcgaggtgccgtaaagcactaaatcggaaccctaaagggagcccccgatttagagcttgacggggaaagccggcgaacgtggcgagaaaggaagggaagaaagcgaaaggagcgggcgctagggcgctggcaagtgtagcggtcacgctgcgcgtaaccaccacacccgccgcgcttaatgcgccgctacagggcgcgtccattcgccattcaggctgcgcaactgttgggaagggcgatcggtgcgggcctcttcgctattacgccagctggcgaaagggggatgtgctgcaaggcgattaagttgggtaacgccagggttttcccagtcacgacgttgtaaaacgacggccagtgaattgtaatacgactcactatagggcgaattgggccctctagatgcatgctcgagcggccgccagtgtgatggatatctgcagaattcgccctttaacagcatgagtgaacagaaccatctctatgatagtcctgaatggctttttggtctgaaaaatatgcattggctctcattacatttaaccaaaattatcacaatataagaatgagatctttaacattgccaattaggtcagtggtcccaagtagtcacttagaaaatctgtgtatgtgaaatactgtttgtgacttaaaatgaaatttatttttaataggtgaacataatattgaggagacagaacatacagagcaaaagcgaaatgtgattcgaattattcctcaccacaactacaatgcagctattaataagtacaaccatgacattgcccttctggaactggacgaacccttagtgctaaacagctacgttacacctatttgcattgctgacaaggaatacacgaacatcttcctcaaatttggatctggctatgtaagtggctggggaagagtcttccacaaagggagatcagctttagttcttcagtaccttagagttccacttgttgaccgagccacatgtcttcgatctacaaagttcaccatctataacaacatgttctgtgctggcttccatgaaggaggtagagattcatgtcaaggagatagtgggggaccccatgttactgaagtggaagggaccagtttcttaactggaattattagctggggtgaagagtgtgcaatgaaaggcaaatatggaatatataccaaggtatcccggtatgtcaactggattaaggaaaaaacaaagctcacttaatgaaagatggatttccaaggttaattcattggaattgaaaattaacagggcctctcactaactaatcactttcccatcttttgttagatttgaatatatacattctatgatcattgctttttctctttacaggggagaatttcatattttacctgagcaaattgattagaaaatggaaccactagaggaatataatgtgttaggaaattacagtcatttctaagggcccagaagggcgaattccagcacactggcggccgttactagtggatccgagctcggtaccaagcttggcgtaatcatggtcatagctgtttcctgtgtgaaattgttatccgctcacaattccacacaacatacgagccggaagcataaagtgtaaagcctggggtgcctaatgagtgagctaactcacattaattgcgttgcgctcactgcccgctttccagtcgggaaacctgtcgtgccagctgcattaatgaatcggccaacgcgcggggagaggcggtttgcgtattgggcgct

SEQ ID NO: 38 - DNA, 6996 bp, Artificial Sequence
  Plasmid pDuoF9-ex8 (outcome)
  P3 binding site (1373)..(1392)
  Recombinase R1 (placeholder) (1519)..(2550)
  Recombinase R#7-B5 (placeholder) (1519)..(2550)
  Ribosome binding site (2551)..(2633)
  LoxF9a (4220)..(4253)
  exchanged part of human F9 gene including exon 8 (4220)..(4253)
  LoxF9b (4962)..(5019)
  P4 binding site (4962)..(4981)
  CmR (5127)..(5786)
  Origin of replication (6148)..(6996)
gctcatgagcccgaagtggcgagcccgatcttccccatcggtgatgtcggcgatataggcgccagcaaccgcacctgtggcgccggtgatgccggccacgatgcgtccggcgtagaggatctgctcatgtttgacagcttatcatcgatgcataatgtgcctgtcaaatggacgaagcagggattctgcaaaccctatgctactccgtcaagccgtcaattgtctgattcgttaccaattatgacaacttgacggctacatcattcactttttcttcacaaccggcacggaactcgctcgggctggccccggtgcattttttaaatacccgcgagaaatagagttgatcgtcaaaaccaacattgcgaccgacggtggcgataggcatccgggtggtgctcaaaagcagcttcgcctggctgatacgttggtcctcgcgccagcttaagacgctaatccctaactgctggcggaaaagatgtgacagacgcgacggcgacaagcaaacatgctgtgcgacgctggcgatatcaaaattgctgtctgccaggtgatcgctgatgtactgacaagcctcgcgtacccgattatccatcggtggatggagcgactcgttaatcgcttccatgcgccgcagtaacaattgctcaagcagatttatcgccagcagctccgaatagcgcccttccccttgcccggcgttaatgatttgcccaaacaggtcgctgaaatgcggctggtgcgcttcatccgggcgaaagaaccccgtattggcaaatattgacggccagttaagccattcatgccagtaggcgcgcggacgaaagtaaacccactggtgataccattcgcgagcctccggatgacgaccgtagtgatgaatctctcctggcgggaacagcaaaatatcacccggtcggcaaacaaattctcgtccctgatttttcaccaccccctgaccgcgaatggtgagattgagaatataacctttcattcccagcggtcggtcgataaaaaaatcgagataaccgttggcctcaatcggcgttaaacccgccaccagatgggcattaaacgagtatcccggcagcaggggatcattttgcgcttcagccatacttttcatactcccgccattcagagaagaaaccaattgtccatattgcatcagacattgccgtcactgcgtcttttactggctcttctcgctaaccaaaccggtaaccccgcttattaaaagcattctgtaacaaagcgggaccaaagccatgacaaaaacgcgtaacaaaagtgtctataatcacggcagaaaagtccacattgattatttgcacggcgtcacactttgctatgccatagcatttttatccataagattagcggatcctacctgacgctttttatcgcaactctctactgtttctccatacccgtttttttgggctagcgaattcgagctctaaggaggtgccacaattctcgagccatacccattctaatgatcataaggaggtgtacatgtcaatactactgaccttgcaccaaagtttgtccgcattactggtcgatgcaacgagtgatgaggctcgcaagaacctgatggatgtgctcagggatcgccaggcgttctccgagcgtacctggaaagtgctcctgtccgtttgccggacgtgggcggcatggtgcaagttgaacaaccggaaatggtttcccgcggaacctgaagatgttcgcgattaccttctacatcttcaggctcgcggtctggcagtaaacactatcctgcaacatttggcccagctaaacatgctccaccgtcggttcgggctgccacgaccgggcgacagcgacgctgtttcactggttatgcggcgaatccgaagggagaacgtcgatgctggtgagcgtaccaagcaggccctagcgttcgagcgcactgacttcgaccaggttcgtgcactcatggaaaatagcgaacggggccaggatatacgtactctggcacttctgggggttgcttataacaccctgttacgcgtatccgaaattgccaggattcggattaaagacatctcacgtactgacggtgggaggatgctaatccacattagcagaacgaaaacgctggtcagcaccgcaggcgtagagaaggcgcttagcctgggggtaactaaactggtcgagcgatggatttccgtctctggtgtggctagtgacccaaacaattacctgttttgccaggttagaataaatggtgtggccgtgccgtctgccaccagccggctatcaaccgacgtcctgcgaaagatttttgaggctgcccaccgcctgatctacggtgccaaggatggctctggtcagagatacctggcctggtctgggcacagtgcccgtgtcggagccgcgcgggatatggcccgcgctggggtttcaatagcggagattatgcaggctggtggctggaccaccgtagagagtgtcatgaactatatccgtaacctggacagtgagacaggggcaatggtgcgtctgctggaagatggcgactagtctagaggtaccattccgatcgcggatcggccggaatgggatagacgtcctatcatccacacctactagttaaggaggtgtacatgtcaatactactgaccttgcaccaaagtttgtccgcattactggtcgatgcaacgagtgatgaggctcgcaagaacctgatggatgtgctcagggatcgccaggcgttctccgagcgtacctggaaagtgctcctgtccgtttgccggacgtgggcggcatggtgcaagttgaacaaccggaaatggtttcccgcggaacctgaagatgttcgcgattaccttctacatcttcaggctcgcggtctggcagtaaacactatcctgcaacatttggcccagctaaacatgctccaccgtcggttcgggctgccacgaccgggcgacagcgacgctgtttcactggttatgcggcgaatccgaagggagaacgtcgatgctggtgagcgtaccaagcaggccctagcgttcgagcgcactgacttcgaccaggttcgtgcactcatggaaaatagcgaacggggccaggatatacgtactctggcacttctgggggttgcttataacaccctgttacgcgtatccgaaattgccaggattcggattaaagacatctcacgtactgacggtgggaggatgctaatccacattagcagaacgaaaacgctggtcagcaccgcaggcgtagagaaggcgcttagcctgggggtaactaaactggtcgagcgatggatttccgtctctggtgtggctagtgacccaaacaattacctgttttgccaggttagaataaatggtgtggccgtgccgtctgccaccagccggctatcaaccgacgtcctgcgaaagatttttgaggctgcccaccgcctgatctacggtgccaaggatggctctggtcagagatacctggcctggtctgggcacagtgcccgtgtcggagccgcgcgggatatggcccgcgctggggtttcaatagcggagattatgcaggctggtggctggaccaccgtagagagtgtcatgaactatatccgtaacctggacagtgagacaggggcaatggtgcgtctgctggaagatggcgactagtctagacgtacgcctgcaggcaagcttggctgttttggcggatgagagaagattttcagcctgatacagattaaatcagaacgcagaagcggtctgataaaacagaatttgcctggcggcagtagcgcggtggtcccacctgaccccatgccgaactcagaagtgaaacgccgtagcgccgatggtagtgtggggtctccccatgcgagagtagggaactgccaggcatcaaataaaacgaaaggctcagtcgaaagactgggcctttcgttttatctgttgtttgtcggtgaacgctctcctgagtaggacaaatccgccgggagcggatttgaacgttgcgaagcaacggcccggagggtggcgggcaggacgcccgccataaactgccaggcatcaaattaagcagaaggccatcctgacggatggcctttttgcgtttctacaaactcttttgtttatttttctaaatacattcaaatatgtatccgctcatgagacaataaccctgataaatgcttcaataatattgaaaaaggaagagtatgagatctctcattacatttaaccaaaattatcacaatataagaatgagatctttaacattgccaattaggtcagtggtcccaagtagtcacttagaaaatctgtgtatgtgaaatactgtttgtgacttaaaatgaaatttatttttaataggtgaacataatattgaggagacagaacatacagagcaaaagcgaaatgtgattcgaattattcctcaccacaactacaatgcagctattaataagtacaaccatgacattgcccttctggaactggacgaacccttagtgctaaacagctacgttacacctatttgcattgctgacaaggaatacacgaacatcttcctcaaatttggatctggctatgtaagtggctggggaagagtcttccacaaagggagatcagctttagttcttcagtaccttagagttccacttgttgaccgagccacatgtcttcgatctacaaagttcaccatctataacaacatgttctgtgctggcttccatgaaggaggtagagattcatgtcaaggagatagtgggggaccccatgttactgaagtggaagggaccagtttcttaactggaattattagctggggtgaagagtgtgcaatgaaaggcaaatatggaatatataccaaggtatcccggtatgtcaactggattaaggaaaaaacaaagctcacttaatgaaagatggatttccaaggttaattcattggaattgaaaattaacagggcctctcactaactaatcactttcccatcttttgttagatttgaatatatacattctaagatctggtcgaatttgctttcgaatttctgccattcatccgcttattatcacttattcaggcgtagcaccaggcgtttaagggcaccaataactgccttaaaaaaattacgccccgccctgccactcatcgcagtactgttgtaattcattaagcattctgccgacatggaagccatcacagacggcatgatgaacctgaatcgccagcggcatcagcaccttgtcgccttgcgtataatatttgcccatggtgaaaacgggggcgaagaagttgtccatattggccacgtttaaatcaaaactggtgaaactcacccagggattggctgagacgaaaaacatattctcaataaaccctttagggaaataggccaggttttcaccgtaacacgccacatcttgcgaatatatgtgtagaaactgccggaaatcgtcgtggtattcactccagagcgatgaaaacgtttcagtttgctcatggaaaacggtgtaacaagggtgaacactatcccatatcaccagctcaccgtctttcattgccatacggaattccggatgagcattcatcaggcgggcaagaatgtgaataaaggccggataaaacttgtgcttatttttctttacggtctttaaaaaggccgtaatatccagctgaacggtctggttataggtacattgagcaactgactgaaatgcctcaaaatgttctttacgatgccattgggatatatcaacggtggtatatccagtgatttttttctccattttagcttccttagctcctgaaaatctcgataactcaaaaaatacgcccggtagtgatcttatttcattatggtgaaagttggaacctcttacgtgccgatcaacgtctcattttcgccaaaagttggcccagggcttcccggtatcaacagggacaccaggatttatttattctgcgaagtgatcttccgtcacaggtatttattcggcgcaaagtgcgtcgggtgatgctgccaacttactgatttagtgtatgatggtgtttttgaggtgctccagtggcttctgtttctatcagctgtccctcctgttcagctactgacggggtggtgcgtaacggcaaaagcaccgccggacatcagcgctagcggagtgtatactggcttactatgttggcactgatgagggtgtcagtgaagtgcttcatgtggcaggagaaaaaaggctgcaccggtgcgtcagcagaatatgtgatacaggatatattccgcttcctcgctcactgactcgctacgctcggtcgttcgactgcggcgagcggaaatggcttacgaacggggcggagatttcctggaagatgccaggaagatacttaacagggaagtgagagggccgcggcaaagccgtttttccataggctccgcccccctgacaagcatcacgaaatctgacgctcaaatcagtggtggcgaaacccgacaggactataaagataccaggcgtttccccctggcggctccctcgtgcgctctcctgttcctgcctttcggtttaccggtgtcattccgctgttatggccgcgtttgtctcattccacgcctgacactcagttccgggtaggcagttcgctccaagctggactgtatgcacgaaccccccgttcagtccgaccgctgcgccttatccggtaactatcgtcttgagtccaacccggaaagacatgcaaaagcaccactggcagcagccactggtaattgatttagaggagttagtcttgaagtcatgcgccggttaaggctaaactgaaaggacaagttttggtgactgcgctcctccaagccagttacctcggttcaaagagttggtagctcagagaaccttcgaaaaaccgccctgcaaggcggttttttcgttttcagagcaagagattacgcgcagaccaaaacgatctcaagaagatcatcttattaatcagataaaatatttctag

SEQ ID NO: 39 - protein, 343 aa, Bacteriophage P1
MSNLLTVHQNLPALPVDATSDEVRKNLMDMFRDRQAFSEHTWKMLLSVCRSWAAWCKLNNRKWFPAEPEDVRDYLLYLQARGLAVKTIQQHLGQLNMLHRRSGLPRPSDSNAVSLVMRRIRKENVDAGERAKQALAFERTDFDQVRSLMENSDRCQDIRNLAFLGIAYNTLLRIAEIARIRVKDISRTDGGRMLIHIGRTKTLVSTAGVEKALSLGVTKLVERWISVSGVADDPNNYLFCRVRKNGVAAPSATSQLSTRALEGIFEATHRLIYGAKDDSGQRYLAWSGHSARVGAARDMARAGVSIPEIMQAGGWTNVNIVMNYIRNLDSETGAMVRLLEDGD

SEQ ID NO: 40 - DNA, 34 bp, Homo sapiens
tacacagtgtatattgatttttatcaaatgcctt

SEQ ID NO: 41 - DNA, 34 bp, Homo sapiens
tacacaatgtatattgatttttatcaaatgcctt

SEQ ID NO: 42 - DNA, 34 bp, Artificial Sequence
  Intermediate target site HexL
tacacagtgtatattgatttttatacattgtgta

SEQ ID NO: 43 - DNA, 34 bp, Artificial Sequence
  Intermediate target site HexR
aaggcatttgatattgatttttatcaaatgcctt

SEQ ID NO: 44 - DNA, 34 bp, Artificial Sequence
  Intermediate target site HexR1
aagacattttatattgatttttataaaatgtctt

SEQ ID NO: 45 - DNA, 34 bp, Artificial Sequence
  Intermediate target site HexR2
aacgcattggatattgatttttatccaatgcgtt

SEQ ID NO: 46 - protein, 343 aa, Artificial Sequence
  Recombinase Hex-R-#7
MSNLQTLHQNLSALLADATSDEARKNLTDVLRDSQAFSEHTWRVLLSVCRSWAAWCELNNRKWFPAEPEDVRDYLLHLQARGLTVNTIQQHLCQLNMLHRRSGLPPPGDSNAASLVMRRIRKENVDAGERVKQALAFERTDLDQVCALMENSNRCQDIRNLAFLGVAYNTLLRISEVARIRVRDITRTDGGRMLIHIGRTKTLVSTAGVEKALSLRVTKLVERWISVSGVADDPNNFLFCRVGRNGVAVSSATSQLSTPALQGIFASAHRLIYGARDDPGQRYLTWSGHSARVGAARDMARAGVPIAEIMQAGGWTTIESVMNYLRNLDSETGAMVRLLEGDD

SEQ ID NO: 47 - protein, 343 aa, Artificial Sequence
  Recombinase Hex-L-#7
MSNLQTLHQNLSALLVDVTSDEARKSLMDMLRDRQAFSEHTWKMLLSVCRSWAAWCESNNRKWFPAEPEDVRDYLLHLQARGLAVRTIQQHLCQLNMLHRRSGLPRPGDSNAVSLVMRRIRKENVDAGERAKQALAFERTDFDQVRSLMEDSDRCQDIRNLAFLGIAYNTLLRISEIARIRVRDISRTDGGRMLIHIGRTKTLISTAGVEKALSLGVTKLVERWISVSGVADDPNNYLFCRVRKHGVAAPSATSQLSTNALQRIFEAAHCLIYGAKDDSGQRYLAWSGHSARVGAARDMARAGVSIPEIMQAGGWTTVNSVMNYIRNLDSETGAMVRLLEEGD

SEQ ID NO: 48 - protein, 343 aa, Artificial Sequence
  Recombinase Hex-R-#30
MSYLHTLHQSLSALLVNATSDEARKNLMDVFRDCQAFSEHTWRVLLSVCRSWVTWCKLNNRKWFPAEPEDVRDYLLHLQARGLTVNTIQQHLCQLNMLHRRSGLPRPGDSNAVTLVMRRIRKENVDAGERTKQALAFERTDFGQVRSLMENSDRCRDIRNLAFLGVAYNTLLRISEIARIRVRDISRTDGGRMLIHIGRTKTLVSTAGAEKALSQGVTKLVERWISVSGVADDPNNYLFCRVRRNGVAAPSATGQLSTPALQGIFVSAHRLVYGARDASGQRYLTWSGHSARVGTARDMARAGVPIAEIMQAGGWTTIESVMNYLRNLDSETGAMVRLLEDDD

SEQ ID NO: 49 - protein, 343 aa, Artificial Sequence
  Recombinase Hex-L-#30
MSNLQTLHQNLSALLVDATCDEARENLLNMFRDRQAFSEHTWKMLLSVCRSWAAWCELNNRKWFPAEPEDVRDYLLHLQARGLAVKTIQQHLAQLNMLHRRSGLPRPGDSNAVSLVVRRIRKENVDAGERAKQALAFERTDFDQVRSLMENSDRCQDIRNLAFLGIAYNTLLRISEIARIRVKDISRTDGGRMLIHIGRTKTLVSTAGVEKALSLGVTKLVERWISVSGVADDPNNYLFCRVSKYGVAAPSATSQLSTHALQRIFEAAHRLIYGAKDDSGRRYLAWSGHSARVGAARDMARAGVSIPEIMQAGGWATVNSVMNYSRNLDSEAGAMVRLLEDGD